European Patent Application EP 4 219 699 A1, published August 2, 2023. Title: ENGINEERING OF SYSTEMS, METHODS AND OPTIMIZED GUIDE COMPOSITIONS WITH NEW ARCHITECTURES FOR SEQUENCE MANIPULATION. Applicant: The Broad Institute, Inc. The sequence listing filed with the application follows.

SEQUENCE LISTING (148 sequences)

SEQ ID NO: 1 - protein, 4 aa, synthetic construct
  REGION 1..4: note = source = /note="Description of Artificial Sequence: Syntheticpeptide"
GGGS

SEQ ID NO: 2 - protein, 12 aa, synthetic construct
  REGION 1..12: note = source = /note="Description of Artificial Sequence: Syntheticpeptide"
GGGSGGGSGGGS

SEQ ID NO: 3 - protein, 7 aa, synthetic construct
  REGION 1..7: note = source = /note="Description of Artificial Sequence: Syntheticpeptide"
AEAAAKA

SEQ ID NO: 4 - protein, 15 aa, synthetic construct
  REGION 1..15: note = source = /note="Description of Artificial Sequence: Syntheticpeptide"
GGGGSGGGGSGGGGS

SEQ ID NO: 5 - protein, 30 aa, synthetic construct
  REGION 1..30: note = source = /note="Description of Artificial Sequence: Syntheticpolypeptide"
GGGGSGGGGSGGGGSGGGGSGGGGSGGGGS

SEQ ID NO: 6 - protein, 45 aa, synthetic construct
  REGION 1..45: note = source = /note="Description of Artificial Sequence: Syntheticpolypeptide"
GGGGSGGGGSGGGGSGGGGSGGGGSGGGGSGGGGSGGGGSGGGGS

SEQ ID NO: 7 - protein, 60 aa, synthetic construct
  REGION 1..60: note = source = /note="Description of Artificial Sequence: Syntheticpolypeptide"
GGGGSGGGGSGGGGSGGGGSGGGGSGGGGSGGGGSGGGGSGGGGSGGGGSGGGGSGGGGS

SEQ ID NO: 8 - protein, 5 aa, synthetic construct
  REGION 1..5: note = source = /note="Description of Artificial Sequence: Syntheticpeptide"
GGGGS

SEQ ID NO: 9 - protein, 10 aa, synthetic construct
  REGION 1..10: note = source = /note="Description of Artificial Sequence: Syntheticpeptide"
GGGGSGGGGS

SEQ ID NO: 10 - protein, 20 aa, synthetic construct
  REGION 1..20: note = source = /note="Description of Artificial Sequence: Syntheticpeptide"
GGGGSGGGGSGGGGSGGGGS

SEQ ID NO: 11 - protein, 25 aa, synthetic construct
  REGION 1..25: note = source = /note="Description of Artificial Sequence: Syntheticpeptide"
GGGGSGGGGSGGGGSGGGGSGGGGS

SEQ ID NO: 12 - protein, 35 aa, synthetic construct
  REGION 1..35: note = source = /note="Description of Artificial Sequence: Syntheticpolypeptide"
GGGGSGGGGSGGGGSGGGGSGGGGSGGGGSGGGGS

SEQ ID NO: 13 - protein, 40 aa, synthetic construct
  REGION 1..40: note = source = /note="Description of Artificial Sequence: Syntheticpolypeptide"
GGGGSGGGGSGGGGSGGGGSGGGGSGGGGSGGGGSGGGGS

SEQ ID NO: 14 - protein, 50 aa, synthetic construct
  REGION 1..50: note = source = /note="Description of Artificial Sequence: Syntheticpolypeptide"
GGGGSGGGGSGGGGSGGGGSGGGGSGGGGSGGGGSGGGGSGGGGSGGGGS

SEQ ID NO: 15 - protein, 55 aa, synthetic construct
  REGION 1..55: note = source = /note="Description of Artificial Sequence: Syntheticpolypeptide"
GGGGSGGGGSGGGGSGGGGSGGGGSGGGGSGGGGSGGGGSGGGGSGGGGSGGGGS

SEQ ID NO: 16 - DNA, 12 bp, synthetic construct
  misc_feature 1..12: note = source = /note="Description of Artificial Sequence: Syntheticoligonucleotide"
  source 1..12: mol_type = other DNA
acttgtttaagt

SEQ ID NO: 17 - skipped

SEQ ID NO: 18 - DNA, 16 bp, synthetic construct
  misc_feature 1..16: note = source = /note="Description of Artificial Sequence: Syntheticoligonucleotide"
  source 1..16: mol_type = other DNA
ggcaccgagtcggtgc

SEQ ID NO: 19 - RNA, 30 nt, synthetic construct
  modified_base 2..5: mod_base = OTHER; note = a, c, u, g, unknown or other
  modified_base 8..20: mod_base = OTHER; note = a, c, u, g, unknown or other
  modified_base 23: mod_base = OTHER; note = a, c, u, g, unknown or other
  misc_feature 1..30: note = See specification as filed for detailed description ofsubstitutions and preferred embodiments
  misc_feature 1..30: note = source = /note="Description of Artificial Sequence: Syntheticoligonucleotide"
  source 1..30: mol_type = other RNA
gnnnnagnnnnnnnnnnnnnaanttrrrrt

SEQ ID NO: 20 - DNA, 20 bp, Homo sapiens
  source 1..20: mol_type = genomic DNA
gagtccgagcagaagaagaa

SEQ ID NO: 21-32 - skipped (12 entries)

SEQ ID NO: 33 - DNA, 137 bp, synthetic construct
  modified_base 1..20: mod_base = OTHER; note = a, c, t, g, unknown or other
  misc_feature 1..137: note = source = /note="Description of Artificial Sequence: Syntheticpolynucleotide"
  source 1..137: mol_type = other DNA
nnnnnnnnnnnnnnnnnnnngtttttgtactctcaagatttagaaataaatcttgcagaagctacaaagataaggcttcatgccgaaatcaacaccctgtcattttatggcagggtgttttcgttatttaatttttt

SEQ ID NO: 34 - DNA, 123 bp, synthetic construct
  modified_base 1..20: mod_base = OTHER; note = a, c, t, g, unknown or other
  misc_feature 1..123: note = source = /note="Description of Artificial Sequence: Syntheticpolynucleotide"
  source 1..123: mol_type = other DNA
nnnnnnnnnnnnnnnnnnnngtttttgtactctcagaaatgcagaagctacaaagataaggcttcatgccgaaatcaacaccctgtcattttatggcagggtgttttcgttatttaatttttt

SEQ ID NO: 35 - DNA, 110 bp, synthetic construct
  modified_base 1..20: mod_base = OTHER; note = a, c, t, g, unknown or other
  misc_feature 1..110: note = source = /note="Description of Artificial Sequence: Syntheticpolynucleotide"
  source 1..110: mol_type = other DNA
nnnnnnnnnnnnnnnnnnnngtttttgtactctcagaaatgcagaagctacaaagataaggcttcatgccgaaatcaacaccctgtcattttatggcagggtgttttttt

SEQ ID NO: 36 - DNA, 102 bp, synthetic construct
  modified_base 1..20: mod_base = OTHER; note = a, c, t, g, unknown or other
  misc_feature 1..102: note = source = /note="Description of Artificial Sequence: Syntheticpolynucleotide"
  source 1..102: mol_type = other DNA
nnnnnnnnnnnnnnnnnnnngttttagagctagaaatagcaagttaaaataaggctagtccgttatcaacttgaaaaagtggcaccgagtcggtgctttttt

SEQ ID NO: 37 - DNA, 88 bp, synthetic construct
  modified_base 1..20: mod_base = OTHER; note = a, c, t, g, unknown or other
  misc_feature 1..88: note = source = /note="Description of Artificial Sequence: Syntheticoligonucleotide"
  source 1..88: mol_type = other DNA
nnnnnnnnnnnnnnnnnnnngttttagagctagaaatagcaagttaaaataaggctagtccgttatcaacttgaaaaagtgttttttt

SEQ ID NO: 38 - DNA, 76 bp, synthetic construct
  modified_base 1..20: mod_base = OTHER; note = a, c, t, g, unknown or other
  misc_feature 1..76: note = source = /note="Description of Artificial Sequence: Syntheticoligonucleotide"
  source 1..76: mol_type = other DNA
nnnnnnnnnnnnnnnnnnnngttttagagctagaaatagcaagttaaaataaggctagtccgttatcatttttttt

SEQ ID NO: 39 - DNA, 20 bp, Homo sapiens
  source 1..20: mol_type = genomic DNA
gagtcctagcaggagaagaa

SEQ ID NO: 40 - DNA, 20 bp, Homo sapiens
  source 1..20: mol_type = genomic DNA
gagtctaagcagaagaagaa

SEQ ID NO: 41 - protein, 7 aa, Simian virus 40
PKKKRKV

SEQ ID NO: 42 - protein, 16 aa, unidentified
  REGION 1..16: note = source = /note="Description of Unknown:Nucleoplasmin bipartite NLS sequence"
KRPAATKKAGQAKKKK

SEQ ID NO: 43 - protein, 9 aa, unidentified
  REGION 1..9: note = source = /note="Description of Unknown:C-myc NLS sequence"
PAAKRVKLD

SEQ ID NO: 44 - protein, 11 aa, unidentified
  REGION 1..11: note = source = /note="Description of Unknown:C-myc NLS sequence"
RQRRNELKRSP

SEQ ID NO: 45 - protein, 38 aa, Homo sapiens
NQSSNFGPMKGGNFGGRSSGPYGGGGQYFAKPRNQGGY

SEQ ID NO: 46 - protein, 42 aa, unidentified
  REGION 1..42: note = source = /note="Description of Unknown:IBB domain from importin-alpha sequence"
RMRIZFKNKGKDTAELRRRRVEVSVELRKAKKDEQILKRRNV

SEQ ID NO: 47 - protein, 8 aa, unidentified
  REGION 1..8: note = source = /note="Description of Unknown:Myoma T protein sequence"
VSRKRPRP

SEQ ID NO: 48 - protein, 8 aa, unidentified
  REGION 1..8: note = source = /note="Description of Unknown:Myoma T protein sequence"
PPKKARED

SEQ ID NO: 49 - protein, 8 aa, Homo sapiens
PQPKKKPL

SEQ ID NO: 50 - protein, 12 aa, Mus musculus
SALIKKKKKMAP

SEQ ID NO: 51 - protein, 5 aa, Influenza virus
DRLRR

SEQ ID NO: 52 - protein, 7 aa, Influenza virus
PKQKKRK

SEQ ID NO: 53 - protein, 10 aa, Hepatitis delta virus
RKLKKKIKKL

SEQ ID NO: 54 - protein, 10 aa, Mus musculus
REKKKFLKRR

SEQ ID NO: 55 - protein, 20 aa, Homo sapiens
KRKGDEVDGVDEVAKKKSKK

SEQ ID NO: 56 - protein, 17 aa, Homo sapiens
RKCLQAGMNLEARKTKK

SEQ ID NO: 57 - RNA, 12 nt, synthetic construct
  misc_feature 1..12: note = source = /note="Description of Artificial Sequence: Syntheticoligonucleotide"
  source 1..12: mol_type = other RNA
gttttagagcta

SEQ ID NO: 58 - RNA, 36 nt, synthetic construct
  misc_feature 1..36: note = source = /note="Description of Artificial Sequence: Syntheticoligonucleotide"
  source 1..36: mol_type = other RNA
gttttagtactctgtaattttaggtatgaggtagac

SEQ ID NO: 59 - RNA, 84 nt, synthetic construct
  misc_feature 1..84: note = source = /note="Description of Artificial Sequence: Syntheticoligonucleotide"
  source 1..84: mol_type = other RNA
ttgtacttatacctaaaattacagaatctactaaaacaaggcaaaatgccgtgtttatctcgtcaacttgttggcgagattttt

SEQ ID NO: 60 - RNA, 80 nt, synthetic construct
  misc_feature 1..80: note = source = /note="Description of Artificial Sequence: Syntheticoligonucleotide"
  source 1..80: mol_type = other RNA
gccccagagctagaaatagcaagttggggtaaggctagtccgttatcaacttgaaaaagtggcaccgagtcggtgctttt

SEQ ID NO: 61 - RNA, 80 nt, synthetic construct
  misc_feature 1..80: note = source = /note="Description of Artificial Sequence: Syntheticoligonucleotide"
  source 1..80: mol_type = other RNA
gttttagagcccgaaagggcaagttaaaataaggctagtccgttatcaacttgaaaaagtggcaccgagtcggtgctttt

SEQ ID NO: 62 - RNA, 76 nt, synthetic construct
  misc_feature 1..76: note = source = /note="Description of Artificial Sequence: Syntheticoligonucleotide"
  source 1..76: mol_type = other RNA
gttttagagcgaaagcaagttaaaataaggctagtccgttatcaacttgaaaaagtggcaccgagtcggtgctttt

SEQ ID NO: 63 - RNA, 74 nt, synthetic construct
  misc_feature 1..74: note = source = /note="Description of Artificial Sequence: Syntheticoligonucleotide"
  source 1..74: mol_type = other RNA
gttttagaggaaacaagttaaaataaggctagtccgttatcaacttgaaaaagtggcaccgagtcggtgctttt

SEQ ID NO: 64 - RNA, 71 nt, synthetic construct
  misc_feature 1..71: note = source = /note="Description of Artificial Sequence: Syntheticoligonucleotide"
  source 1..71: mol_type = other RNA
gttttagagacaagttaaaataaggctagtccgttatcaacttgaaaaagtggcaccgagtcggtgctttt

SEQ ID NO: 65 - RNA, 78 nt, synthetic construct
  misc_feature 1..78: note = source = /note="Description of Artificial Sequence: Syntheticoligonucleotide"
  source 1..78: mol_type = other RNA
gttttagagctagaaatagctttaaaataaggctagtccgttatcaacttgaaaaagtggcaccgagtcggtgctttt

SEQ ID NO: 66 - RNA, 78 nt, synthetic construct
  misc_feature 1..78: note = source = /note="Description of Artificial Sequence: Syntheticoligonucleotide"
  source 1..78: mol_type = other RNA
gttttagcgctagaaatagcgttaaaataaggctagtccgttatcaacttgaaaaagtggcaccgagtcggtgctttt

SEQ ID NO: 67 - RNA, 80 nt, synthetic construct
  misc_feature 1..80: note = source = /note="Description of Artificial Sequence: Syntheticoligonucleotide"
  source 1..80: mol_type = other RNA
gttttagcgctagaaatagcaagttaaaataaggctagtccgttatcaacttgaaaaagtggcaccgagtcggtgctttt

SEQ ID NO: 68 - RNA, 80 nt, synthetic construct
  misc_feature 1..80: note = source = /note="Description of Artificial Sequence: Syntheticoligonucleotide"
  source 1..80: mol_type = other RNA
gttttagtgctagaaatagcaagttaaaataaggctagtccgttatcaacttgaaaaagtggcaccgagtcggtgctttt

SEQ ID NO: 69 - RNA, 80 nt, synthetic construct
  misc_feature 1..80: note = source = /note="Description of Artificial Sequence: Syntheticoligonucleotide"
  source 1..80: mol_type = other RNA
gttttagggctagaaatagcaagttaaaataaggctagtccgttatcaacttgaaaaagtggcaccgagtcggtgctttt

SEQ ID NO: 70 - RNA, 80 nt, synthetic construct
  misc_feature 1..80: note = source = /note="Description of Artificial Sequence: Syntheticoligonucleotide"
  source 1..80: mol_type = other RNA
gttttagagctagaaatagcttgttaaaataaggctagtccgttatcaacttgaaaaagtggcaccgagtcggtgctttt

SEQ ID NO: 71 - RNA, 80 nt, synthetic construct
  misc_feature 1..80: note = source = /note="Description of Artificial Sequence: Syntheticoligonucleotide"
  source 1..80: mol_type = other RNA
gttttagagctagaaatagcaacttaaaataaggctagtccgttatcaacttgaaaaagtggcaccgagtcggtgctttt

SEQ ID NO: 72 - RNA, 80 nt, synthetic construct
  misc_feature 1..80: note = source = /note="Description of Artificial Sequence: Syntheticoligonucleotide"
  source 1..80: mol_type = other RNA
gttttagagctagaaatagcaaattaaaataaggctagtccgttatcaacttgaaaaagtggcaccgagtcggtgctttt

SEQ ID NO: 73 - RNA, 80 nt, synthetic construct
  misc_feature 1..80: note = source = /note="Description of Artificial Sequence: Syntheticoligonucleotide"
  source 1..80: mol_type = other RNA
gttttagagctagaaatagcaatttaaaataaggctagtccgttatcaacttgaaaaagtggcaccgagtcggtgctttt

SEQ ID NO: 74 - RNA, 80 nt, synthetic construct
  misc_feature 1..80: note = source = /note="Description of Artificial Sequence: Syntheticoligonucleotide"
  source 1..80: mol_type = other RNA
gttttagagctagaaatagcaagttaaaataattctagtaagttatcaacttgaaaaagtggcaccgagtcggtgctttt

SEQ ID NO: 75 - RNA, 76 nt, synthetic construct
  misc_feature 1..76: note = source = /note="Description of Artificial Sequence: Syntheticoligonucleotide"
  source 1..76: mol_type = other RNA
gttttagagctagaaatagcaagttaaaataaggctagtccgtaacttgaaaaagtggcaccgagtcggtgctttt

SEQ ID NO: 76 - RNA, 80 nt, synthetic construct
  misc_feature 1..80: note = source = /note="Description of Artificial Sequence: Syntheticoligonucleotide"
  source 1..80: mol_type = other RNA
gttttagagctagaaatagcaagttaaaataaggctagtccgtatagaacttgaaaaagtggcaccgagtcggtgctttt

SEQ ID NO: 77 - RNA, 80 nt, synthetic construct
  misc_feature 1..80: note = source = /note="Description of Artificial Sequence: Syntheticoligonucleotide"
  source 1..80: mol_type = other RNA
gttttagagctagaaatagcaagttaaaataaggctagtccgttatcacgccgaaaggcgggcaccgagtcggtgctttt

SEQ ID NO: 78 - RNA, 84 nt, synthetic construct
  misc_feature 1..84: note = source = /note="Description of Artificial Sequence: Syntheticoligonucleotide"
  source 1..84: mol_type = other RNA
gttttagagctagaaatagcaagttaaaataaggctagtccgttatcaacttgagaaatcaagtggcaccgagtcggtgctttt

SEQ ID NO: 79 - RNA, 88 nt, synthetic construct
  misc_feature 1..88: note = source = /note="Description of Artificial Sequence: Syntheticoligonucleotide"
  source 1..88: mol_type = other RNA
gttttagagctagaaatagcaagttaaaataaggctagtccgttatcacgccggccgaaaggccggcgggcaccgagtcggtgctttt

SEQ ID NO: 80 - RNA, 80 nt, synthetic construct
  misc_feature 1..80: note = source = /note="Description of Artificial Sequence: Syntheticoligonucleotide"
  source 1..80: mol_type = other RNA
gttttagagctagaaatagcaagttaaaataaggctagtccgttatcaacttaaagaagtggcaccgagtcggtgctttt

SEQ ID NO: 81 - RNA, 80 nt, synthetic construct
  misc_feature 1..80: note = source = /note="Description of Artificial Sequence: Syntheticoligonucleotide"
  source 1..80: mol_type = other RNA
gttttagagctagaaatagcaagttaaaataaggctagtccgttatcaacttgaaaaagtggccccgcggcggggctttt

SEQ ID NO: 82 - RNA, 82 nt, synthetic construct
  misc_feature 1..82: note = source = /note="Description of Artificial Sequence: Syntheticoligonucleotide"
  source 1..82: mol_type = other RNA
gttttagagctagaaatagcaagttaaaataaggctagtccgttatcaacttgaaaaagtggcaccgaagttcggtgctttt

SEQ ID NO: 83 - RNA, 84 nt, synthetic construct
  misc_feature 1..84: note = source = /note="Description of Artificial Sequence: Syntheticoligonucleotide"
  source 1..84: mol_type = other RNA
gttttagagctagaaatagcaagttaaaataaggctagtccgttatcaacttgaaaaagtggcaccgaaagtttcggtgctttt

SEQ ID NO: 84 - RNA, 84 nt, synthetic construct; identical to SEQ ID NO: 83
  misc_feature 1..84: note = source = /note="Description of Artificial Sequence: Syntheticoligonucleotide"
  source 1..84: mol_type = other RNA

SEQ ID NO: 85 - RNA, 80 nt, synthetic construct
  misc_feature 1..80: note = source = /note="Description of Artificial Sequence: Syntheticoligonucleotide"
  source 1..80: mol_type = other RNA
gttttagagctagaaatagcaagctaaaataaggctagtccgttatcaacttgaaaaagtggcaccgagtcggtgctttt

SEQ ID NO: 86 - RNA, 80 nt, synthetic construct
  misc_feature 1..80: note = source = /note="Description of Artificial Sequence: Syntheticoligonucleotide"
  source 1..80: mol_type = other RNA
gttttagatctagaaatagcaaggtaaaataaggctagtccgttatcaacttgaaaaagtggcaccgagtcggtgctttt

SEQ ID NO: 87 - RNA, 80 nt, synthetic construct
  misc_feature 1..80: note = source = /note="Description of Artificial Sequence: Syntheticoligonucleotide"
  source 1..80: mol_type = other RNA
gttttagagctagaaatagcaagataaaataaggctagtccgttatcaacttgaaaaagtggcaccgagtcggtgctttt

SEQ ID NO: 88 - RNA, 80 nt, synthetic construct
  misc_feature 1..80: note = source = /note="Description of Artificial Sequence: Syntheticoligonucleotide"
  source 1..80: mol_type = other RNA
gttttagagctagaaatagcaagttaaaacaaggctagtccgttatcaacttgaaaaagtggcaccgagtcggtgctttt

SEQ ID NO: 89 - RNA, 80 nt, synthetic construct
  misc_feature 1..80: note = source = /note="Description of Artificial Sequence: Syntheticoligonucleotide"
  source 1..80: mol_type = other RNA
tttttagagctagaaatagcaagttaaaagaaggctagtccgttatcaacttgaaaaagtggcaccgagtcggtgctttt

SEQ ID NO: 90 - RNA, 80 nt, synthetic construct
  misc_feature 1..80: note = source = /note="Description of Artificial Sequence: Syntheticoligonucleotide"
  source 1..80: mol_type = other RNA
gttttagagctagaaatagcaagttaaaaaaaggctagtccgttatcaacttgaaaaagtggcaccgagtcggtgctttt

SEQ ID NO: 91 - RNA, 80 nt, synthetic construct
  misc_feature 1..80: note = source = /note="Description of Artificial Sequence: Syntheticoligonucleotide"
  source 1..80: mol_type = other RNA
gttttagagctagaaatagcaagttaaaataaggctagaccgttatcaacttgaaaaagtggcaccgagtcggtgctttt

SEQ ID NO: 92 - RNA, 80 nt, synthetic construct
  misc_feature 1..80: note = source = /note="Description of Artificial Sequence: Syntheticoligonucleotide"
  source 1..80: mol_type = other RNA
gttttagagctagaaatagcaagttaaaataaggctagcccgttatcaacttgaaaaagtggcaccgagtcggtgctttt

SEQ ID NO: 93 - RNA, 80 nt, synthetic construct
  misc_feature 1..80: note = source = /note="Description of Artificial Sequence: Syntheticoligonucleotide"
  source 1..80: mol_type = other RNA
gttttagagctagaaatagcaagttaaaataaggctagtccgttatcaacttgaaaaagtggcaccgaatcggtgctttt

SEQ ID NO: 94 - RNA, 80 nt, synthetic construct
  misc_feature 1..80: note = source = /note="Description of Artificial Sequence: Syntheticoligonucleotide"
  source 1..80: mol_type = other RNA
gttttagagctagaaatagcaagttaaaataaggctagtccgttatcaacttgaaaaagtggcaccgactcggtgctttt

SEQ ID NO: 95 - RNA, 80 nt, synthetic construct
  misc_feature 1..80: note = source = /note="Description of Artificial Sequence: Syntheticoligonucleotide"
  source 1..80: mol_type = other RNA
gttttagagctagaaatagcaagttaaaataaggctagtccgttatcaacttgaaaaagtggcaccgattcggtgctttt

SEQ ID NO: 96 - RNA, 80 nt, synthetic construct
  misc_feature 1..80: note = source = /note="Description of Artificial Sequence: Syntheticoligonucleotide"
  source 1..80: mol_type = other RNA
gttttagagctagaaatagcaagttaaaataaggctagtccgttatcaacttgaaaaagtggcaccgagacggtgctttt

SEQ ID NO: 97 - RNA, 80 nt, synthetic construct
  misc_feature 1..80: note = source = /note="Description of Artificial Sequence: Syntheticoligonucleotide"
  source 1..80: mol_type = other RNA
gttttagagctagaaatagcaagttaaaataaggctagtccgttatcaacttgaaaaagtggcaccgagccggtgctttt

SEQ ID NO: 98 - RNA, 80 nt, synthetic construct
  misc_feature 1..80: note = source = /note="Description of Artificial Sequence: Syntheticoligonucleotide"
  source 1..80: mol_type = other RNA
gttttagagctagaaatagcaagttaaaataaggctagtccgttatcaacttgaaaaagtggcaccgagtcggtgctttt

SEQ ID NO: 99 - RNA, 80 nt, synthetic construct; identical to SEQ ID NO: 98
  misc_feature 1..80: note = source = /note="Description of Artificial Sequence: Syntheticoligonucleotide"
  source 1..80: mol_type = other RNA

SEQ ID NO: 100 - RNA, 81 nt, synthetic construct
  misc_feature 1..81: note = source = /note="Description of Artificial Sequence: Syntheticoligonucleotide"
  source 1..81: mol_type = other RNA
gccccagagctagaaatagcaaagttggggtaaggctagtccgttatcaacttgaaaaagtggcaccgagtcggtgctttt

SEQ ID NO: 101 - RNA, 80 nt, synthetic construct
  misc_feature 1..80: note = source = /note="Description of Artificial Sequence: Syntheticoligonucleotide"
  source 1..80: mol_type = other RNA
gggggagagctagaaatagcaagttcccctaaggctagtccgttatcaacttgaaaaagtggcaccgagtcggtgctttt

SEQ ID NO: 102 - RNA, 78 nt, synthetic construct
  misc_feature 1..78: note = source = /note="Description of Artificial Sequence: Syntheticoligonucleotide"
  source 1..78: mol_type = other RNA
gtttagagctagaaatagcaagttaaataaggctagtccgttatcaacttgaaaaagtggcaccgagtcggtgctttt

SEQ ID NO: 103 - RNA, 76 nt, synthetic construct
  misc_feature 1..76: note = source = /note="Description of Artificial Sequence: Syntheticoligonucleotide"
  source 1..76: mol_type = other RNA
gttagagctagaaatagcaagttaataaggctagtccgttatcaacttgaaaaagtggcaccgagtcggtgctttt

SEQ ID NO: 104 - RNA, 86 nt, synthetic construct
  misc_feature 1..86: note = source = /note="Description of Artificial Sequence: Syntheticoligonucleotide"
  source 1..86: mol_type = other RNA
gttttagagctagaaatagcaagttaaaataaggctagtccgttatcaacttgaaaaagtggcaccgaaaagttttcggtgctttt

SEQ ID NO: 105 - RNA, 76 nt, synthetic construct
  misc_feature 1..76: note = source = /note="Description of Artificial Sequence: Syntheticoligonucleotide"
  source 1..76: mol_type = other RNA
gccccagagctagaaatagcaagttggggtaaggctagtccgtaacttgaaaaagtggcaccgagtcggtgctttt

SEQ ID NO: 106 - RNA, 80 nt, synthetic construct
  misc_feature 1..80: note = source = /note="Description of Artificial Sequence: Syntheticoligonucleotide"
  source 1..80: mol_type = other RNA
gccccagcgctagaaatagcaagttggggtaaggctagtccgttatcacgccgaaaggcgggcaccgagtcggtgctttt

SEQ ID NO: 107 - RNA, 80 nt, synthetic construct
  misc_feature 1..80: note = source = /note="Description of Artificial Sequence: Syntheticoligonucleotide"
  source 1..80: mol_type = other RNA
gccccagggctagaaatagcaagttggggtaaggctagtccgttatcacgccgaaaggcgggcaccgagtcggtgctttt

SEQ ID NO: 108 - RNA, 69 nt, synthetic construct
  misc_feature 1..69: note = source = /note="Description of Artificial Sequence: Syntheticoligonucleotide"
  source 1..69: mol_type = other RNA
gttttagagacaagttaaaataaggctagtccgtacgccgaaaggcgggcaccgacggtcggtgctttt

SEQ ID NO: 109 - RNA, 69 nt, synthetic construct; identical to SEQ ID NO: 108
  misc_feature 1..69: note = source = /note="Description of Artificial Sequence: Syntheticoligonucleotide"
  source 1..69: mol_type = other RNA

SEQ ID NO: 110 - RNA, 47 nt, synthetic construct
  misc_feature 1..47: note = source = /note="Description of Artificial Sequence: Syntheticoligonucleotide"
  source 1..47: mol_type = other RNA
gttttagagctagaaatagcaagttaaaataaggctagtccgttttt

SEQ ID NO: 111 - RNA, 56 nt, synthetic construct
  misc_feature 1..56: note = source = /note="Description of Artificial Sequence: Syntheticoligonucleotide"
  source 1..56: mol_type = other RNA
gttttagagctagaaatagcaagttaaaataaggctagtccgttatcatttttttt

SEQ ID NO: 112 - RNA, 68 nt, synthetic construct
  misc_feature 1..68: note = source = /note="Description of Artificial Sequence: Syntheticoligonucleotide"
  source 1..68: mol_type = other RNA
gttttagagctagaaatagcaagttaaaataaggctagtccgttatcaacttgaaaaagtgttttttt

SEQ ID NO: 113 - RNA, 82 nt, synthetic construct
  misc_feature 1..82: note = source = /note="Description of Artificial Sequence: Syntheticoligonucleotide"
  source 1..82: mol_type = other RNA
gttttagagctagaaatagcaagttaaaataaggctagtccgttatcaacttgaaaaagtggcaccgagtcggtgctttttt

SEQ ID NO: 114 - RNA, 81 nt, synthetic construct
  misc_feature 1..81: note = source = /note="Description of Artificial Sequence: Syntheticoligonucleotide"
  source 1..81: mol_type = other RNA
gttttagagctagaaatagcaaggtaaaataaggctagtccgttatcaacttgaaaaagtggcaccgagtcggtgcttttt

SEQ ID NO: 115 - RNA, 80 nt, synthetic construct
  misc_feature 1..80: note = source = /note="Description of Artificial Sequence: Syntheticoligonucleotide"
  source 1..80: mol_type = other RNA
gccccagagctaattatagcaagttggggtaaggctagtccgttatcacgccaccaggcgggcaccgagtcggtgctttt

SEQ ID NO: 116 - RNA, 76 nt, synthetic construct
  misc_feature 1..76: note = source = /note="Description of Artificial Sequence: Syntheticoligonucleotide"
  source 1..76: mol_type = other RNA
gccccagagcattagcaagttggggtaaggctagtccgttatcacgccaccaggcgggcaccgagtcggtgctttt

SEQ ID NO: 117 - RNA, 71 nt, synthetic construct
  misc_feature 1..71: note = source = /note="Description of Artificial Sequence: Syntheticoligonucleotide"
  source 1..71: mol_type = other RNA
gccccagagacaagttggggtaaggctagtccgttatcacgccaccaggcgggcaccgagtcggtgctttt

SEQ ID NO: 118 - RNA, 78 nt, synthetic construct
  misc_feature 1..78: note = source = /note="Description of Artificial Sequence: Syntheticoligonucleotide"
  source 1..78: mol_type = other RNA
gccccagagcattagcaagttggggtaaggctagtccgttatcacgccaccaggcgccgcggcagtgccgcggttttt

SEQ ID NO: 119 - RNA, 78 nt, synthetic construct
  misc_feature 1..78: note = source = /note="Description of Artificial Sequence: Syntheticoligonucleotide"
  source 1..78: mol_type = other RNA
gccccagcgcattagcaagttggggtaaggctagtccgttatcacgccaccaggcgccgcggcagtgccgcggttttt

SEQ ID NO: 120 - RNA, 72 nt, synthetic construct
  misc_feature 1..72: note = source = /note="Description of Artificial Sequence: Syntheticoligonucleotide"
  source 1..72: mol_type = other RNA
gccccagagcattagcaagttggggtaaggctagtccgttatcacgccaccaggcgccgcagtgcggttttt

SEQ ID NO: 121 - RNA, 82 nt, synthetic construct
  misc_feature 1..82: note = source = /note="Description of Artificial Sequence: Syntheticoligonucleotide"
  source 1..82: mol_type = other RNA
gccccagagcattagcaagttggggtaaggctagtccgttatcacgccaccaggcgccgcggcgcagtgcgccgcggttttt

SEQ ID NO: 122 - RNA, 80 nt, synthetic construct
  misc_feature 1..80: note = source = /note="Description of Artificial Sequence: Syntheticoligonucleotide"
  source 1..80: mol_type = other RNA
gttttagagctagaaatagcaagttaaaataagccatgtgcgttatcaacttgaaaaagtggcaccgagtcggtgctttt

SEQ ID NO: 123 - RNA, 76 nt, synthetic construct
  misc_feature 1..76: note = source = /note="Description of Artificial Sequence: Syntheticoligonucleotide"
  source 1..76: mol_type = other RNA
gccccagagcattagcaagttggggtaagccatgtgcgttatcagggcaccagcccggcaccgagtcggtgctttt

SEQ ID NO: 124 - RNA, 78 nt, synthetic construct
  misc_feature 1..78: note = source = /note="Description of Artificial Sequence: Syntheticoligonucleotide"
  source 1..78: mol_type = other RNA
gccccagagcattagcaagttggggtaagccatgtgcgttatcagggcaccagcccccgcggcagtgccgcggttttt

SEQ ID NO: 125 - RNA, 80 nt, synthetic construct; identical to SEQ ID NO: 76
  misc_feature 1..80: note = source = /note="Description of Artificial Sequence: Syntheticoligonucleotide"
  source 1..80: mol_type = other RNA

SEQ ID NO: 126 - RNA, 76 nt, synthetic construct
  misc_feature 1..76: note = source = /note="Description of Artificial Sequence: Syntheticoligonucleotide"
  source 1..76: mol_type = other RNA
gccccagagcattagcaagttggggtaaggctagtccgtatagacgccaccaggcgggcaccgagtcggtgctttt

SEQ ID NO: 127 - RNA, 79 nt, synthetic construct
  misc_feature 1..79: note = source = /note="Description of Artificial Sequence: Syntheticoligonucleotide"
  source 1..79: mol_type = other RNA
agccccagagcattagcaagttggggtaaggctagtccgtatagacgccaccaggcgccgcggcagtgccgcggttttt

SEQ ID NO: 128 - RNA, 80 nt, synthetic construct
  misc_feature 1..80: note = source = /note="Description of Artificial Sequence: Syntheticoligonucleotide"
  source 1..80: mol_type = other RNA
gttttagagctagaaatagcaagttaaaattagccatgtgcgtatagaacttgaaaaagtggcaccgattcggtgctttt

SEQ ID NO: 129 - RNA, 76 nt, synthetic construct
  misc_feature 1..76: note = source = /note="Description of Artificial Sequence: Syntheticoligonucleotide"
  source 1..76: mol_type = other RNA
gccccagagcattagcaagttggggttagccatgtgcgtatagagggcaccagcccggcaccgattcggtgctttt

SEQ ID NO: 130 - RNA, 78 nt, synthetic construct
  misc_feature 1..78: note = source = /note="Description of Artificial Sequence: Syntheticoligonucleotide"
  source 1..78: mol_type = other RNA
gccccagagcattagcaagttggggttagccatgtgcgtatagagggcaccagcccccgcggcattgccgcggttttt

SEQ ID NO: 131 - RNA, 78 nt, synthetic construct
  misc_feature 1..78: note = source = /note="Description of Artificial Sequence: Syntheticoligonucleotide"
  source 1..78: mol_type = other RNA
gccccagccgattacgaagttggggttagccatgtgcgtatagagggcaccagcccccgcggcattgccgcggttttt

SEQ ID NO: 132 - RNA, 78 nt, synthetic construct
  misc_feature 1..78: note = source = /note="Description of Artificial Sequence: Syntheticoligonucleotide"
  source 1..78: mol_type = other RNA
gccccagccgattacgaagttggggcttgccatgtgcggatagtgggcaccagcccccgcggcattgccgcggttttt

SEQ ID NO: 133 - RNA, 148 nt, synthetic construct
  modified_base 1..21: mod_base = OTHER; note = a, c, u, g, unknown or other
  misc_feature 1..148: note = source = /note="Description of Artificial Sequence: Syntheticpolynucleotide"
  source 1..148: mol_type = other RNA
nnnnnnnnnnnnnnnnnnnnngttttagtactctgtaattttaggtatgaggtagacgaaaattgtacttatacctaaaattacagaatctactaaaacaaggcaaaatgccgtgtttatctcgtcaacttgttggcgagattttttt

SEQ ID NO: 134 - RNA, 126 nt, synthetic construct
  modified_base 1..21: mod_base = OTHER; note = a, c, u, g, unknown or other
  misc_feature 1..126: note = source = /note="Description of Artificial Sequence: Syntheticpolynucleotide"
  source 1..126: mol_type = other RNA
nnnnnnnnnnnnnnnnnnnnngttttagtactctgtaattttaggtgaaaacctaaaattacagaatctactaaaacaaggcaaaatgccgtgtttatctcgtcaacttgttggcgagattttttt

SEQ ID NO: 135 - RNA, 118 nt, synthetic construct
  modified_base 1..21: mod_base = OTHER; note = a, c, u, g, unknown or other
  misc_feature 1..118: note = source = /note="Description of Artificial Sequence: Syntheticpolynucleotide"
  source 1..118: mol_type = other RNA
nnnnnnnnnnnnnnnnnnnnngttttagtactctgtaattttgaaaaaaattacagaatctactaaaacaaggcaaaatgccgtgtttatctcgtcaacttgttggcgagattttttt

SEQ ID NO: 136 - RNA, 112 nt, synthetic construct
  modified_base 1..21: mod_base = OTHER; note = a, c, u, g, unknown or other
  misc_feature 1..112: note = source = /note="Description of Artificial Sequence: Syntheticpolynucleotide"
  source 1..112: mol_type = other RNA
nnnnnnnnnnnnnnnnnnnnngttttagtactctgtaatgaaaattacagaatctactaaaacaaggcaaaatgccgtgtttatctcgtcaacttgttggcgagattttttt

SEQ ID NO: 137 - RNA, 106 nt, synthetic construct
  modified_base 1..21: mod_base = OTHER; note = a, c, u, g, unknown or other
  misc_feature 1..106: note = source = /note="Description of Artificial Sequence: Syntheticpolynucleotide"
  source 1..106: mol_type = other RNA
nnnnnnnnnnnnnnnnnnnnngttttagtactctgtgaaaacagaatctactaaaacaaggcaaaatgccgtgtttatctcgtcaacttgttggcgagattttttt

SEQ ID NO: 138 - RNA, 104 nt, synthetic construct
  modified_base 1..21: mod_base = OTHER; note = a, c, u, g, unknown or other
  misc_feature 1..104: note = source = /note="Description of Artificial Sequence: Syntheticpolynucleotide"
  source 1..104: mol_type = other RNA
nnnnnnnnnnnnnnnnnnnnngttttagtactctggaaacagaatctactaaaacaaggcaaaatgccgtgtttatctcgtcaacttgttggcgagattttttt

SEQ ID NO: 139-140 - skipped (2 entries)

SEQ ID NO: 141 - DNA, 27 bp, synthetic construct
  modified_base 21..27: mod_base = OTHER; note = a, c, t, g, unknown or other
  misc_feature 1..27: note = source = /note="Description of Artificial Sequence: Syntheticoligonucleotide"
  source 1..27: mol_type = other DNA
gggactcaaccaagtcattcnnnnnnn

SEQ ID NO: 142 - DNA, 27 bp, synthetic construct
  modified_base 1..7: mod_base = OTHER; note = a, c, t, g, unknown or other
  misc_feature 1..27: note = source = /note="Description of Artificial Sequence: Syntheticoligonucleotide"
  source 1..27: mol_type = other DNA
nnnnnnngaatgacttggttgagtccc

SEQ ID NO: 143 - RNA, 20 nt, synthetic construct
  misc_feature 1..20: note = source = /note="Description of Artificial Sequence: Syntheticoligonucleotide"
  source 1..20: mol_type = other RNA
gggactcaaccaagtcattc

SEQ ID NO: 144 - DNA, 27 bp, synthetic construct
  misc_feature 1..27: note = source = /note="Description of Artificial Sequence: Syntheticoligonucleotide"
  source 1..27: mol_type = other DNA
ggcctccccaaagcctggccagggagt

SEQ ID NO: 145 - DNA, 27 bp, synthetic construct
  misc_feature 1..27: note = source = /note="Description of Artificial Sequence: Syntheticoligonucleotide"
  source 1..27: mol_type = other DNA
tggccaggctttggggaggcctggagt

SEQ ID NO: 146 - RNA, 46 nt, synthetic construct
  misc_feature 1..46: note = source = /note="Description of Artificial Sequence: Syntheticoligonucleotide"
  source 1..46: mol_type = other RNA
gttttagagctagaaatagcaagttaaaataaggctagtccgtttt

SEQ ID NO: 147 - RNA, 65 nt, synthetic construct
  misc_feature 1..65: note = source = /note="Description of Artificial Sequence: Syntheticoligonucleotide"
  source 1..65: mol_type = other RNA
gttttagagctagaaatagcaagttaaaataaggctagtccgttatcaacttgaaaaagtgtttt

SEQ ID NO: 148 - RNA, 80 nt, synthetic construct
  misc_feature 1..80: note = source = /note="Description of Artificial Sequence: Syntheticoligonucleotide"
  source 1..80: mol_type = other RNA
gttttagagctagaaatagcaaggtaaaataaggctagtccgttatcaacttgaaaaagtggcaccgagtcggtgctttt